European Patent Application EP 4 257 676 A1, published October 11, 2023. Title: 修饰的免疫细胞及其用途. Applicant: 北京卡替医疗技术有限公司. The sequence listing filed with the application follows.

SEQUENCE LISTING (4 sequences)

SEQ ID NO: 1 - DNA, 705 bp, Artificial Sequence
  Enhanced receptor V1E coding sequence
atgcagatcccacaggcgccctggccagtcgtctgggcggtgctacaactgggctggcggccaggatggttcttagactccccagacaggccctggaacccccccaccttctccccagccctgctcgtggtgaccgaaggggacaacgccaccttcacctgcagcttctccaacacatcggagagcttcgtgctaaactggtaccgcatgagccccagcaaccagacggacaagctggccgccttccccgaggaccgcagccagcccggccaggactgccgcttccgtgtcacacaactgcccaacgggcgtgacttccacatgagcgtggtcagggcccggcgcaatgacagcggcacctacctctgtggggccatctccctggcccccaaggcgcagatcaaagagagcctgcgggcagagctcagggtgacagagagaagggcagaagtgcccacagcccactgtccaagtcccctatttcccggaccttctaagcccttttgggtgctggtggtggttggtggagtcctggcttgctatagcttgctagtaacagtggcctttattattttctgggtgaggagtaagaggagcaggctcctgcacagtgactacatgaacatgactccccgccgccccgggcccacccgcaagcattaccagccctatgccccaccacgcgacttcgcagcctatcgctcc

SEQ ID NO: 2 - DNA, 1023 bp, Artificial Sequence
  Enhanced receptor V2E coding sequence
atggccttaccagtgaccgccttgctcctgccgctggccttgctgctccacgccgccaggccggacatccagatgacccagagccctagcagcctgagcgctagcgtgggagatagagtgaccatcacctgcagggcctctcaggatgtgtctacagccgtggcttggtaccagcagaagccaggaaaggcccccaagctgctgatctacagcgcctctttcctgtacagcggcgtgcctagcagattcagcggcagcggaagcggcaccgatttcaccctgaccatcagcagcctgcagccagaggacttcgccacctactactgccagcagtacctgtaccacccagccaccttcggacagggcaccaaggtggagatcaagggtggcggtggctcgggcggtggtgggtcgggtggcggcggatctgaggtgcagctggtggaatcaggaggaggactggtgcagccaggaggatctctgagactgtcttgcgccgccagcggctttacattcagcgactcttggatccattgggtgcgccaggctccaggaaaaggactcgagtgggtggcttggatcagcccttacggcggcagcacctactacgccgatagcgtgaagggcaggttcaccatcagcgccgataccagcaagaacaccgcctacctgcagatgaacagcctgagggccgaggataccgccgtgtactattgcgccaggaggcattggccaggcggatttgactattggggccagggaacactggtgaccgtgtccagctgtccaagtcccctatttcccggaccttctaagcccttttgggtgctggtggtggttggtggagtcctggcttgctatagcttgctagtaacagtggcctttattattttctgggtgaggagtaagaggagcaggctcctgcacagtgactacatgaacatgactccccgccgccccgggcccacccgcaagcattaccagccctatgccccaccacgcgacttcgcagcctatcgctcc

SEQ ID NO: 3 - DNA, 1467 bp, Artificial Sequence
  CD19 CAR coding sequence
atgggctggtcttgcatcatcctgttcctcgtggccaccgccaccggcgtccacagcgccatccagctcacccagagcccctcgagcttgagtgcctcggtgggagaccgggtcactatcacctgccgagccagtcagggcatctcctccgcccttgcctggtaccagcagaagcccgggaaggcccccaagctgctgatctacgacgctagtagtctggagagtggcgtgccttcgcgcttctcgggcagtgggagtggcaccgacttcaccttgaccatctccagtctacagccggaagatttcgcgacctactactgtcagcaattcaactcttatccatacactttcggccaggggacaaagctggagatcaagggcgggggcgggagtggcggcggagggtccggaggcgggggctccgaggtgcaactagtccagagcggagccgaggtgaagaagcccggggagagtctaaagatctcttgcaagggctccggttactccttctcgagttcctggatcgggtgggtgcgacagatgccgggcaagggcctggagtggatgggcattatctaccccgacgactccgatacccgttatagtccatcgttccagggacaggtgaccatttccgccgacaagtctatcagaaccgcctatctgcagtggtccagtctgaaggcctctgacactgccatgtattattgcgccaggcacgttacgatgatctggggggtgatcatcgacttctggggccagggcacactcgtaaccgtcagttctgcggccgcaaccacgacgccagcgccgcgaccaccaacaccggcgcccaccatcgcgtcgcagcccctgtccctgcgcccagaggcgtgccggccagcggcggggggcgcagtgcacacgagggggctggacttcgcctgtgatatctacatctgggcgcccttggccgggacttgtggggtccttctcctgtcactggttatcaccctttactgcaaacggggcagaaagaaactcctgtatatattcaaacaaccatttatgagaccagtacaaactactcaagaggaagatggctgtagctgccgatttccagaagaagaagaaggaggatgtgaactgagagtgaagttcagcaggagcgcagacgcccccgcgtacaagcagggccagaaccagctctataacgagctcaatctaggacgaagagaggagtacgacgttttggacaagagacgtggccgggaccctgagatggggggaaagccgagaaggaagaaccctcaggaaggcctgtacaatgaactgcagaaagataagatggcggaggcctacagtgagattgggatgaaaggcgagcgccggaggggcaaggggcacgatggcctttaccagggtctcagtacagccaccaaggacacctacgacgcccttcacatgcaggccctgccccctcgctaa

SEQ ID NO: 4 - DNA, 20 bp, Artificial Sequence
  sgRNA for knocking out PD-1
gtctgggcggtgctacaact